European Patent Application EP 4 223 129 A1, published August 9, 2023. Title: MUTANT TRANSGLUTAMINASE. Applicant: Ajinomoto Co., Inc. The sequence listing filed with the application follows.

SEQUENCE LISTING (114 sequences)

SEQ ID NO: 1 - DNA, 996 bp, Streptoverticillium mobaraense
gactccgacgacagggtcacccctcccgccgagccgctcgacaggatgcccgacccgtaccgtccctcgtacggcagggccgagacggtcgtcaacaactacatacgcaagtggcagcaggtctacagccaccgcgacggcaggaagcagcagatgaccgaggagcagcgggagtggctgtcctacggctgcgtcggtgtcacctgggtcaattcgggtcagtacccgacgaacagactggccttcgcgtccttcgacgaggacaggttcaagaacgagctgaagaacggcaggccccggtccggcgagacgcgggcggagttcgagggccgcgtcgcgaaggagagcttcgacgaggagaagggcttccagcgggcgcgtgaggtggcgtccgtcatgaacagggccctggagaacgcccacgacgagagcgcttacctcgacaacctcaagaaggaactggcgaacggcaacgacgccctgcgcaacgaggacgcccgttccccgttctactcggcgctgcggaacacgccgtccttcaaggagcggaacggaggcaatcacgacccgtccaggatgaaggccgtcatctactcgaagcacttctggagcggccaggaccggtcgagttcggccgacaagaggaagtacggcgacccggacgccttccgccccgccccgggcaccggcctggtcgacatgtcgagggacaggaacattccgcgcagccccaccagccccggtgagggattcgtcaatttcgactacggctggttcggcgcccagacggaagcggacgccgacaagaccgtctggacccacggaaatcactatcacgcgcccaatggcagcctgggtgccatgcatgtctacgagagcaagttccgcaactggtccgagggttactcggacttcgaccgcggagcctatgtgatcaccttcatccccaagagctggaacaccgcccccgacaaggtaaagcagggctggccgtga

SEQ ID NO: 2 - protein, 331 aa, Streptoverticillium mobaraense
DSDDRVTPPAEPLDRMPDPYRPSYGRAETVVNNYIRKWQQVYSHRDGRKQQMTEEQREWLSYGCVGVTWVNSGQYPTNRLAFASFDEDRFKNELKNGRPRSGETRAEFEGRVAKESFDEEKGFQRAREVASVMNRALENAHDESAYLDNLKKELANGNDALRNEDARSPFYSALRNTPSFKERNGGNHDPSRMKAVIYSKHFWSGQDRSSSADKRKYGDPDAFRPAPGTGLVDMSRDRNIPRSPTSPGEGFVNFDYGWFGAQTEADADKTVWTHGNHYHAPNGSLGAMHVYESKFRNWSEGYSDFDRGAYVITFIPKSWNTAPDKVKQGWP

SEQ ID NO: 3 - DNA, 1131 bp, Streptoverticillium mobaraense
gacaatggcgcgggggaagagacgaagtcctacgccgaaacctaccgcctcacggcggatgacgtcgcgaacatcaacgcgctcaacgaaagcgctccggccgcttcgagcgccggcccgtcgttccgggcccccgactccgacgacagggtcacccctcccgccgagccgctcgacaggatgcccgacccgtaccgtccctcgtacggcagggccgagacggtcgtcaacaactacatacgcaagtggcagcaggtctacagccaccgcgacggcaggaagcagcagatgaccgaggagcagcgggagtggctgtcctacggctgcgtcggtgtcacctgggtcaattcgggtcagtacccgacgaacagactggccttcgcgtccttcgacgaggacaggttcaagaacgagctgaagaacggcaggccccggtccggcgagacgcgggcggagttcgagggccgcgtcgcgaaggagagcttcgacgaggagaagggcttccagcgggcgcgtgaggtggcgtccgtcatgaacagggccctggagaacgcccacgacgagagcgcttacctcgacaacctcaagaaggaactggcgaacggcaacgacgccctgcgcaacgaggacgcccgttccccgttctactcggcgctgcggaacacgccgtccttcaaggagcggaacggaggcaatcacgacccgtccaggatgaaggccgtcatctactcgaagcacttctggagcggccaggaccggtcgagttcggccgacaagaggaagtacggcgacccggacgccttccgccccgccccgggcaccggcctggtcgacatgtcgagggacaggaacattccgcgcagccccaccagccccggtgagggattcgtcaatttcgactacggctggttcggcgcccagacggaagcggacgccgacaagaccgtctggacccacggaaatcactatcacgcgcccaatggcagcctgggtgccatgcatgtctacgagagcaagttccgcaactggtccgagggttactcggacttcgaccgcggagcctatgtgatcaccttcatccccaagagctggaacaccgcccccgacaaggtaaagcagggctggccgtga

SEQ ID NO: 4 - protein, 376 aa, Streptoverticillium mobaraense
DNGAGEETKSYAETYRLTADDVANINALNESAPAASSAGPSFRAPDSDDRVTPPAEPLDRMPDPYRPSYGRAETVVNNYIRKWQQVYSHRDGRKQQMTEEQREWLSYGCVGVTWVNSGQYPTNRLAFASFDEDRFKNELKNGRPRSGETRAEFEGRVAKESFDEEKGFQRAREVASVMNRALENAHDESAYLDNLKKELANGNDALRNEDARSPFYSALRNTPSFKERNGGNHDPSRMKAVIYSKHFWSGQDRSSSADKRKYGDPDAFRPAPGTGLVDMSRDRNIPRSPTSPGEGFVNFDYGWFGAQTEADADKTVWTHGNHYHAPNGSLGAMHVYESKFRNWSEGYSDFDRGAYVITFIPKSWNTAPDKVKQGWP

SEQ ID NO: 5 - DNA, 21 bp, Artificial Sequence
  primer
gggagcagtccttgtgcgctt

SEQ ID NO: 6 - DNA, 21 bp, Artificial Sequence
  primer
acaaggactgctcccaaagat

SEQ ID NO: 7 - DNA, 28 bp, Artificial Sequence
  primer
ggcgaacgccaacgacgccctgcgcaac

SEQ ID NO: 8 - DNA, 28 bp, Artificial Sequence
  primer
tcgttggcgttcgccagttccttcttga

SEQ ID NO: 9 - DNA, 29 bp, Artificial Sequence
  primer
ggcgaactccaacgacgccctgcgcaacg

SEQ ID NO: 10 - DNA, 28 bp, Artificial Sequence
  primer
tcgttggagttcgccagttccttcttga

SEQ ID NO: 11 - DNA, 29 bp, Artificial Sequence
  primer
ggcgaaccgcaacgacgccctgcgcaacg

SEQ ID NO: 12 - DNA, 28 bp, Artificial Sequence
  primer
tcgttgcggttcgccagttccttcttga

SEQ ID NO: 13 - DNA, 29 bp, Artificial Sequence
  primer
ccaggacgagtcgagttcggccgacaaga

SEQ ID NO: 14 - DNA, 28 bp, Artificial Sequence
  primer
ctcgactcgtcctggccgctccagaagt

SEQ ID NO: 15 - DNA, 29 bp, Artificial Sequence
  primer
ggtgagaacttcgtcaatttcgactacgg

SEQ ID NO: 16 - DNA, 29 bp, Artificial Sequence
  primer
gacgaagttctcaccggggctggtggggc

SEQ ID NO: 17 - DNA, 28 bp, Artificial Sequence
  primer
cggtgagagattcgtcaatttcgactac

SEQ ID NO: 18 - DNA, 28 bp, Artificial Sequence
  primer
acgaatctctcaccggggctggtggggc

SEQ ID NO: 19 - DNA, 29 bp, Artificial Sequence
  primer
ggtgagtccttcgtcaatttcgactacgg

SEQ ID NO: 20 - DNA, 29 bp, Artificial Sequence
  primer
gacgaaggactcaccggggctggtggggc

SEQ ID NO: 21 - DNA, 28 bp, Artificial Sequence
  primer
acccacgcaaatcactatcacgcgccca

SEQ ID NO: 22 - DNA, 28 bp, Artificial Sequence
  primer
gtgatttgcgtgggtccagacggtcttg

SEQ ID NO: 23 - DNA, 32 bp, Artificial Sequence
  primer
cgttcgcgcccttcttctccgacgacagggtc

SEQ ID NO: 24 - DNA, 32 bp, Artificial Sequence
  primer
gaccctgtcgtcggagaagaagggcgcgaacg

SEQ ID NO: 25 - DNA, 31 bp, Artificial Sequence
  primer
cgtaccgtccctcgaacggcagggccgagac

SEQ ID NO: 26 - DNA, 31 bp, Artificial Sequence
  primer
gtctcggccctgccgttcgagggacggtacg

SEQ ID NO: 27 - DNA, 31 bp, Artificial Sequence
  primer
cgtaccgtccctcgggcggcagggccgagac

SEQ ID NO: 28 - DNA, 31 bp, Artificial Sequence
  primer
gtctcggccctgccgcccgagggacggtacg

SEQ ID NO: 29 - DNA, 31 bp, Artificial Sequence
  primer
gccaccgcgacggcaagaagcagcagatgac

SEQ ID NO: 30 - DNA, 31 bp, Artificial Sequence
  primer
gtcatctgctgcttcttgccgtcgcggtggc

SEQ ID NO: 31 - DNA, 31 bp, Artificial Sequence
  primer
gccaccgcgacggcatcaagcagcagatgac

SEQ ID NO: 32 - DNA, 31 bp, Artificial Sequence
  primer
gtcatctgctgcttgatgccgtcgcggtggc

SEQ ID NO: 33 - DNA, 32 bp, Artificial Sequence
  primer
gcaggccccggtccaacgagacgcgggcggag

SEQ ID NO: 34 - DNA, 32 bp, Artificial Sequence
  primer
ctccgcccgcgtctcgttggaccggggcctgc

SEQ ID NO: 35 - DNA, 30 bp, Artificial Sequence
  primer
cagggccctggagtccgcccacgacgagag

SEQ ID NO: 36 - DNA, 30 bp, Artificial Sequence
  primer
ctctcgtcgtgggcggactccagggccctg

SEQ ID NO: 37 - DNA, 33 bp, Artificial Sequence
  primer
ctggagaacgcccacgccgagagcgcttacctc

SEQ ID NO: 38 - DNA, 33 bp, Artificial Sequence
  primer
gaggtaagcgctctcggcgtgggcgttctccag

SEQ ID NO: 39 - DNA, 33 bp, Artificial Sequence
  primer
gacgagagcgcttactgggacaacctcaagaag

SEQ ID NO: 40 - DNA, 33 bp, Artificial Sequence
  primer
cttcttgaggttgtcccagtaagcgctctcgtc

SEQ ID NO: 41 - DNA, 32 bp, Artificial Sequence
  primer
ctcgacaacctcaagaccgaactggcgaacgg

SEQ ID NO: 42 - DNA, 32 bp, Artificial Sequence
  primer
ccgttcgccagttcggtcttgaggttgtcgag

SEQ ID NO: 43 - DNA, 30 bp, Artificial Sequence
  primer
ggaactggcgaacaagaacgacgccctgcg

SEQ ID NO: 44 - DNA, 30 bp, Artificial Sequence
  primer
cgcagggcgtcgttcttgttcgccagttcc

SEQ ID NO: 45 - DNA, 31 bp, Artificial Sequence
  primer
gcaacgaggacgccggttccccgttctactc

SEQ ID NO: 46 - DNA, 31 bp, Artificial Sequence
  primer
gagtagaacggggaaccggcgtcctcgttgc

SEQ ID NO: 47 - DNA, 31 bp, Artificial Sequence
  primer
ctcggcgctgcgggacacgccgtccttcaag

SEQ ID NO: 48 - DNA, 31 bp, Artificial Sequence
  primer
cttgaaggacggcgtgtcccgcagcgccgag

SEQ ID NO: 49 - DNA, 30 bp, Artificial Sequence
  primer
cacgccgtccttccgcgagcggaacggagg

SEQ ID NO: 50 - DNA, 30 bp, Artificial Sequence
  primer
cctccgttccgctcgcggaaggacggcgtg

SEQ ID NO: 51 - DNA, 33 bp, Artificial Sequence
  primer
cgccgtccttcaaggatcggaacggaggcaatc

SEQ ID NO: 52 - DNA, 33 bp, Artificial Sequence
  primer
gattgcctccgttccgatccttgaaggacggcg

SEQ ID NO: 53 - DNA, 32 bp, Artificial Sequence
  primer
ggaacggaggcaattacgacccgtccaggatg

SEQ ID NO: 54 - DNA, 32 bp, Artificial Sequence
  primer
catcctggacgggtcgtaattgcctccgttcc

SEQ ID NO: 55 - DNA, 31 bp, Artificial Sequence
  primer
cggaggcaatcacatcccgtccaggatgaag

SEQ ID NO: 56 - DNA, 31 bp, Artificial Sequence
  primer
cttcatcctggacgggatgtgattgcctccg

SEQ ID NO: 57 - DNA, 33 bp, Artificial Sequence
  primer
cattccgcgcagccccgccagccccggtgaggg

SEQ ID NO: 58 - DNA, 33 bp, Artificial Sequence
  primer
ccctcaccggggctggcggggctgcgcggaatg

SEQ ID NO: 59 - DNA, 32 bp, Artificial Sequence
  primer
cgcgcagccccaccaaccccggtgagggattc

SEQ ID NO: 60 - DNA, 32 bp, Artificial Sequence
  primer
gaatccctcaccggggttggtggggctgcgcg

SEQ ID NO: 61 - DNA, 32 bp, Artificial Sequence
  primer
cgcgcagccccacccgccccggtgagggattc

SEQ ID NO: 62 - DNA, 32 bp, Artificial Sequence
  primer
gaatccctcaccggggcgggtggggctgcgcg

SEQ ID NO: 63 - DNA, 32 bp, Artificial Sequence
  primer
cgcgcagccccaccaagcccggtgagggattc

SEQ ID NO: 64 - DNA, 32 bp, Artificial Sequence
  primer
gaatccctcaccgggcttggtggggctgcgcg

SEQ ID NO: 65 - DNA, 31 bp, Artificial Sequence
  primer
ccgtctggacccacgcaaatcactatcacgc

SEQ ID NO: 66 - DNA, 31 bp, Artificial Sequence
  primer
gcgtgatagtgatttgcgtgggtccagacgg

SEQ ID NO: 67 - DNA, 31 bp, Artificial Sequence
  primer
cacgcgcccaatggcccactgggtgccatgc

SEQ ID NO: 68 - DNA, 31 bp, Artificial Sequence
  primer
gcatggcacccagtgggccattgggcgcgtg

SEQ ID NO: 69 - DNA, 32 bp, Artificial Sequence
  primer
gcctgggtgccatgattgtctacgagagcaag

SEQ ID NO: 70 - DNA, 32 bp, Artificial Sequence
  primer
cttgctctcgtagacaatcatggcacccaggc

SEQ ID NO: 71 - DNA, 32 bp, Artificial Sequence
  primer
gcaactggtccgagtggtactcggacttcgac

SEQ ID NO: 72 - DNA, 32 bp, Artificial Sequence
  primer
gtcgaagtccgagtaccactcggaccagttgc

SEQ ID NO: 73 - DNA, 31 bp, Artificial Sequence
  primer
cccccgacaaggtattccagggctggccgtg

SEQ ID NO: 74 - DNA, 31 bp, Artificial Sequence
  primer
cacggccagccctggaataccttgtcggggg

SEQ ID NO: 75 - DNA, 28 bp, Artificial Sequence
  primer
gcctattgcatcaccttcatccccaaga

SEQ ID NO: 76 - DNA, 28 bp, Artificial Sequence
  primer
gcgaagcacagtctgttcgtcgggtact

SEQ ID NO: 77 - DNA, 28 bp, Artificial Sequence
  primer
cagactgtgcttcgcgtccttcgacgag

SEQ ID NO: 78 - DNA, 28 bp, Artificial Sequence
  primer
ggtgatgcaataggctccgcggtcgaag

SEQ ID NO: 79 - DNA, 28 bp, Artificial Sequence
  primer
ggccgctgcgcgaaggagagcttcgacg

SEQ ID NO: 80 - DNA, 28 bp, Artificial Sequence
  primer
cttcaggcagttcttgaacctgtcctcg

SEQ ID NO: 81 - DNA, 28 bp, Artificial Sequence
  primer
aagaactgcctgaagaacggcaggcccc

SEQ ID NO: 82 - DNA, 28 bp, Artificial Sequence
  primer
cttcgcgcagcggccctcgaactccgcc

SEQ ID NO: 83 - DNA, 28 bp, Artificial Sequence
  primer
tcggcctgcaagaggaagtacggcgacc

SEQ ID NO: 84 - DNA, 28 bp, Artificial Sequence
  primer
gaactcgcaccgcgtctcgccgggccgg

SEQ ID NO: 85 - DNA, 28 bp, Artificial Sequence
  primer
acgcggtgcgagttcgagggccgcgtcg

SEQ ID NO: 86 - DNA, 28 bp, Artificial Sequence
  primer
cctcttgcaggccgaactcgactcgtcc

SEQ ID NO: 87 - DNA, 28 bp, Artificial Sequence
  primer
aggaagtgcggcgacccggacgccttcc

SEQ ID NO: 88 - DNA, 28 bp, Artificial Sequence
  primer
ctcgaagcacgcccgcgtctcgccgggc

SEQ ID NO: 89 - DNA, 28 bp, Artificial Sequence
  primer
cgggcgtgcttcgagggccgcgtcgcga

SEQ ID NO: 90 - DNA, 28 bp, Artificial Sequence
  primer
gtcgccgcacttcctcttgtcggccgaa

SEQ ID NO: 91 - DNA, 28 bp, Artificial Sequence
  primer
gccccgtgcaccggcctggtcgacatgt

SEQ ID NO: 92 - DNA, 28 bp, Artificial Sequence
  primer
gcgcaggcagtcgttgcggttcgccagt

SEQ ID NO: 93 - DNA, 28 bp, Artificial Sequence
  primer
aacgactgcctgcgcaacgaggacgccc

SEQ ID NO: 94 - DNA, 28 bp, Artificial Sequence
  primer
gccggtgcacggggcggggcggaaggcg

SEQ ID NO: 95 - DNA, 31 bp, Artificial Sequence
  primer
gactggccttcgcgtgcttcgacgaggacag

SEQ ID NO: 96 - DNA, 31 bp, Artificial Sequence
  primer
ctgtcctcgtcgaagcacgcgaaggccagtc

SEQ ID NO: 97 - DNA, 31 bp, Artificial Sequence
  primer
gcttcgacgaggagtgcggcttccagcgggc

SEQ ID NO: 98 - DNA, 31 bp, Artificial Sequence
  primer
gcccgctggaagccgcactcctcgtcgaagc

SEQ ID NO: 99 - DNA, 32 bp, Artificial Sequence
  primer
cagtacccgacgaactgcctggccttcgcgtc

SEQ ID NO: 100 - DNA, 32 bp, Artificial Sequence
  primer
gacgcgaaggccaggcagttcgtcgggtactg

SEQ ID NO: 101 - DNA, 33 bp, Artificial Sequence
  primer
gaggacgcccgttcctgcttctactcggcgctg

SEQ ID NO: 102 - DNA, 33 bp, Artificial Sequence
  primer
cagcgccgagtagaagcaggaacgggcgtcctc

SEQ ID NO: 103 - DNA, 31 bp, Artificial Sequence
  primer
cgagggccgcgtctgcaaggagagcttcgac

SEQ ID NO: 104 - DNA, 31 bp, Artificial Sequence
  primer
gtcgaagctctccttgcagacgcggccctcg

SEQ ID NO: 105 - DNA, 31 bp, Artificial Sequence
  primer
ggaagtacggcgactgcgacgccttccgccc

SEQ ID NO: 106 - DNA, 31 bp, Artificial Sequence
  primer
gggcggaaggcgtcgcagtcgccgtacttcc

SEQ ID NO: 107 - DNA, 31 bp, Artificial Sequence
  primer
ggagagcttcgactgcgagaagggcttccag

SEQ ID NO: 108 - DNA, 31 bp, Artificial Sequence
  primer
ctggaagcccttctcgcagtcgaagctctcc

SEQ ID NO: 109 - DNA, 31 bp, Artificial Sequence
  primer
gttccgcaactggtgcgagggttactcggac

SEQ ID NO: 110 - DNA, 31 bp, Artificial Sequence
  primer
gtccgagtaaccctcgcaccagttgcggaac

SEQ ID NO: 111 - DNA, 32 bp, Artificial Sequence
  primer
ccttcgacgaggactgcttcaagaacgagctg

SEQ ID NO: 112 - DNA, 32 bp, Artificial Sequence
  primer
cagctcgttcttgaagcagtcctcgtcgaagg

SEQ ID NO: 113 - DNA, 32 bp, Artificial Sequence
  primer
gcgtcgcgaaggagtgcttcgacgaggagaag

SEQ ID NO: 114 - DNA, 32 bp, Artificial Sequence
  primer
cttctcctcgtcgaagcactccttcgcgacgc